European Patent Application EP 4 613 779 A1, published September 10, 2025. Title: CD24 BINDING PROTEIN AND USE THEREOF. Applicant: ACROIMMUNE BIOPHARMA CO., LTD. The sequence listing filed with the application follows.

SEQUENCE LISTING (53 sequences)

SEQ ID NO: 1 - protein, 514 aa, synthetic construct
  REGION 1..514: note = CAR-C1
EVQFVESGGGLVQPGGSLKLSCAASGVTFSEAWMDWVRQASGKGLEWVAEIRDKPNSYVTYYAESVKGRFTISRDDSKSTAYLQMNSLKTEDTAIYYCTGAMDYWGQGTLVTVSSGGGGSGGGGSGGGGSDIVMTQTPLSLSVTIGQPASISCKSSQSLLYSNGKTYLNWLLQKPGQSPKRLIYQVSKLDPGIPDRFSGSGSETDFTLKISRVEAEDVGIYYCMQGSSLPWTFGGGTKVEIKRSVTVSSAAAIEVMYPPPYLDNEKSNGTIIHVKGKHLCPSPLFPGPSKPFWVLVVVGGVLACYSLLVTVAFIIFWVRSKRSRLLHSDYMNMTPRRPGPTRKHYQPYAPPRDFAAYRSKRGRKKLLYIFKQPFMRPVQTTQEEDGCSCRFPEEEEGGCELRVKFSRSADAPAYQQGQNQLYNELNLGRREEYDVLDKRRGRDPEMGGKPQRRKNPQEGLYNELQKDKMAEAYSEIGMKGERRRGKGHDGLYQGLSTATKDTYDALHMQALPPR

SEQ ID NO: 2 - protein, 517 aa, synthetic construct
  REGION 1..517: note = CAR-C2
EVKFEESGGGLVQPGGSIKLSCAASGVTFSEAWMDWVRQSPEKGLEWVAEIRDKPNSYVTYYAESVKGRFTISRDDSKSRVYLQMNNLRTEDTGIYYCTGAMDYWGQGTSVTVSSGSTGGGGSGGGGSGGGGSDIVMTQTPLSLSVTIGQPASISCKSSQSLLYSNGKTYLNWLQQRPGQSPKRLIYQVSKLDPGIPDRFSGSGSETDFTLKISRVEAEDLGIYYCMQGSSLPWTFGGGTKLEIKRSVTVSSAAAIEVMYPPPYLDNEKSNGTIIHVKGKHLCPSPLFPGPSKPFWVLVVVGGVLACYSLLVTVAFIIFWVRSKRSRLLHSDYMNMTPRRPGPTRKHYQPYAPPRDFAAYRSKRGRKKLLYIFKQPFMRPVQTTQEEDGCSCRFPEEEEGGCELRVKFSRSADAPAYQQGQNQLYNELNLGRREEYDVLDKRRGRDPEMGGKPQRRKNPQEGLYNELQKDKMAEAYSEIGMKGERRRGKGHDGLYQGLSTATKDTYDALHMQALPPR

SEQ ID NO: 3 - protein, 524 aa, synthetic construct
  REGION 1..524: note = CAR-C3
EVQFVESGGGLVQPGGSLKLSCAASGVTFSEAWMDWVRQASGKGLEWVAEIRDKPNSYVTYYAESVKGRFTISRDDSKSTAYLQMNSLKTEDTAIYYCTGAMDYWGQGTLVTVSSGGGGSGGGGSGGGGSDIVMTQTPLSLSVTIGQPASISCKSSQSLLYSNGKTYLNWLLQKPGQSPKRLIYQVSKLDPGIPDRFSGSGSETDFTLKISRVEAEDVGIYYCMQGSSLPWTFGGGTKVEIKASSHFVPVFLPAKPTTTPAPRPPTPAPTIASQPLSLRPEACRPAAGGAVHTRGLDFACDFWVLVVVGGVLACYSLLVTVAFIIFWVRSKRSRLLHSDYMNMTPRRPGPTRKHYQPYAPPRDFAAYRSKRGRKKLLYIFKQPFMRPVQTTQEEDGCSCRFPEEEEGGCELRVKFSRSADAPAYQQGQNQLYNELNLGRREEYDVLDKRRGRDPEMGGKPQRRKNPQEGLYNELQKDKMAEAYSEIGMKGERRRGKGHDGLYQGLSTATKDTYDALHMQALPPR

SEQ ID NO: 4 - protein, 527 aa, synthetic construct
  REGION 1..527: note = CAR-C4
EVKFEESGGGLVQPGGSIKLSCAASGVTFSEAWMDWVRQSPEKGLEWVAEIRDKPNSYVTYYAESVKGRFTISRDDSKSRVYLQMNNLRTEDTGIYYCTGAMDYWGQGTSVTVSSGSTGGGGSGGGGSGGGGSDIVMTQTPLSLSVTIGQPASISCKSSQSLLYSNGKTYLNWLQQRPGQSPKRLIYQVSKLDPGIPDRFSGSGSETDFTLKISRVEAEDLGIYYCMQGSSLPWTFGGGTKLEIKASSHFVPVFLPAKPTTTPAPRPPTPAPTIASQPLSLRPEACRPAAGGAVHTRGLDFACDFWVLVVVGGVLACYSLLVTVAFIIFWVRSKRSRLLHSDYMNMTPRRPGPTRKHYQPYAPPRDFAAYRSKRGRKKLLYIFKQPFMRPVQTTQEEDGCSCRFPEEEEGGCELRVKFSRSADAPAYQQGQNQLYNELNLGRREEYDVLDKRRGRDPEMGGKPQRRKNPQEGLYNELQKDKMAEAYSEIGMKGERRRGKGHDGLYQGLSTATKDTYDALHMQALPPR

SEQ ID NO: 5 - protein, 472 aa, synthetic construct
  REGION 1..472: note = CAR-C5
EVQFVESGGGLVQPGGSLKLSCAASGVTFSEAWMDWVRQASGKGLEWVAEIRDKPNSYVTYYAESVKGRFTISRDDSKSTAYLQMNSLKTEDTAIYYCTGAMDYWGQGTLVTVSSGGGGSGGGGSGGGGSDIVMTQTPLSLSVTIGQPASISCKSSQSLLYSNGKTYLNWLLQKPGQSPKRLIYQVSKLDPGIPDRFSGSGSETDFTLKISRVEAEDVGIYYCMQGSSLPWTFGGGTKVEIKRSVTVSSAAAIEVMYPPPYLDNEKSNGTIIHVKGKHLCPSPLFPGPSKPFWVLVVVGGVLACYSLLVTVAFIIFWVRSKRSRLLHSDYMNMTPRRPGPTRKHYQPYAPPRDFAAYRSRVKFSRSADAPAYQQGQNQLYNELNLGRREEYDVLDKRRGRDPEMGGKPQRRKNPQEGLYNELQKDKMAEAYSEIGMKGERRRGKGHDGLYQGLSTATKDTYDALHMQALPPR

SEQ ID NO: 6 - protein, 475 aa, synthetic construct
  REGION 1..475: note = CAR-C6
EVKFEESGGGLVQPGGSIKLSCAASGVTFSEAWMDWVRQSPEKGLEWVAEIRDKPNSYVTYYAESVKGRFTISRDDSKSRVYLQMNNLRTEDTGIYYCTGAMDYWGQGTSVTVSSGSTGGGGSGGGGSGGGGSDIVMTQTPLSLSVTIGQPASISCKSSQSLLYSNGKTYLNWLQQRPGQSPKRLIYQVSKLDPGIPDRFSGSGSETDFTLKISRVEAEDLGIYYCMQGSSLPWTFGGGTKLEIKRSVTVSSAAAIEVMYPPPYLDNEKSNGTIIHVKGKHLCPSPLFPGPSKPFWVLVVVGGVLACYSLLVTVAFIIFWVRSKRSRLLHSDYMNMTPRRPGPTRKHYQPYAPPRDFAAYRSRVKFSRSADAPAYQQGQNQLYNELNLGRREEYDVLDKRRGRDPEMGGKPQRRKNPQEGLYNELQKDKMAEAYSEIGMKGERRRGKGHDGLYQGLSTATKDTYDALHMQALPPR

SEQ ID NO: 7 - protein, 482 aa, synthetic construct
  REGION 1..482: note = CAR-C7
EVQFVESGGGLVQPGGSLKLSCAASGVTFSEAWMDWVRQASGKGLEWVAEIRDKPNSYVTYYAESVKGRFTISRDDSKSTAYLQMNSLKTEDTAIYYCTGAMDYWGQGTLVTVSSGGGGSGGGGSGGGGSDIVMTQTPLSLSVTIGQPASISCKSSQSLLYSNGKTYLNWLLQKPGQSPKRLIYQVSKLDPGIPDRFSGSGSETDFTLKISRVEAEDVGIYYCMQGSSLPWTFGGGTKVEIKASSHFVPVFLPAKPTTTPAPRPPTPAPTIASQPLSLRPEACRPAAGGAVHTRGLDFACDFWVLVVVGGVLACYSLLVTVAFIIFWVRSKRSRLLHSDYMNMTPRRPGPTRKHYQPYAPPRDFAAYRSRVKFSRSADAPAYQQGQNQLYNELNLGRREEYDVLDKRRGRDPEMGGKPQRRKNPQEGLYNELQKDKMAEAYSEIGMKGERRRGKGHDGLYQGLSTATKDTYDALHMQALPPR

SEQ ID NO: 8 - protein, 485 aa, synthetic construct
  REGION 1..485: note = CAR-C8
EVKFEESGGGLVQPGGSIKLSCAASGVTFSEAWMDWVRQSPEKGLEWVAEIRDKPNSYVTYYAESVKGRFTISRDDSKSRVYLQMNNLRTEDTGIYYCTGAMDYWGQGTSVTVSSGSTGGGGSGGGGSGGGGSDIVMTQTPLSLSVTIGQPASISCKSSQSLLYSNGKTYLNWLQQRPGQSPKRLIYQVSKLDPGIPDRFSGSGSETDFTLKISRVEAEDLGIYYCMQGSSLPWTFGGGTKLEIKASSHFVPVFLPAKPTTTPAPRPPTPAPTIASQPLSLRPEACRPAAGGAVHTRGLDFACDFWVLVVVGGVLACYSLLVTVAFIIFWVRSKRSRLLHSDYMNMTPRRPGPTRKHYQPYAPPRDFAAYRSRVKFSRSADAPAYQQGQNQLYNELNLGRREEYDVLDKRRGRDPEMGGKPQRRKNPQEGLYNELQKDKMAEAYSEIGMKGERRRGKGHDGLYQGLSTATKDTYDALHMQALPPR

SEQ ID NO: 9 - protein, 473 aa, synthetic construct
  REGION 1..473: note = CAR-C9
EVQFVESGGGLVQPGGSLKLSCAASGVTFSEAWMDWVRQASGKGLEWVAEIRDKPNSYVTYYAESVKGRFTISRDDSKSTAYLQMNSLKTEDTAIYYCTGAMDYWGQGTLVTVSSGGGGSGGGGSGGGGSDIVMTQTPLSLSVTIGQPASISCKSSQSLLYSNGKTYLNWLLQKPGQSPKRLIYQVSKLDPGIPDRFSGSGSETDFTLKISRVEAEDVGIYYCMQGSSLPWTFGGGTKVEIKRSVTVSSAAAIEVMYPPPYLDNEKSNGTIIHVKGKHLCPSPLFPGPSKPFWVLVVVGGVLACYSLLVTVAFIIFWVKRGRKKLLYIFKQPFMRPVQTTQEEDGCSCRFPEEEEGGCELRVKFSRSADAPAYQQGQNQLYNELNLGRREEYDVLDKRRGRDPEMGGKPQRRKNPQEGLYNELQKDKMAEAYSEIGMKGERRRGKGHDGLYQGLSTATKDTYDALHMQALPPR

SEQ ID NO: 10 - protein, 476 aa, synthetic construct
  REGION 1..476: note = CAR-C10
EVKFEESGGGLVQPGGSIKLSCAASGVTFSEAWMDWVRQSPEKGLEWVAEIRDKPNSYVTYYAESVKGRFTISRDDSKSRVYLQMNNLRTEDTGIYYCTGAMDYWGQGTSVTVSSGSTGGGGSGGGGSGGGGSDIVMTQTPLSLSVTIGQPASISCKSSQSLLYSNGKTYLNWLQQRPGQSPKRLIYQVSKLDPGIPDRFSGSGSETDFTLKISRVEAEDLGIYYCMQGSSLPWTFGGGTKLEIKRSVTVSSAAAIEVMYPPPYLDNEKSNGTIIHVKGKHLCPSPLFPGPSKPFWVLVVVGGVLACYSLLVTVAFIIFWVKRGRKKLLYIFKQPFMRPVQTTQEEDGCSCRFPEEEEGGCELRVKFSRSADAPAYQQGQNQLYNELNLGRREEYDVLDKRRGRDPEMGGKPQRRKNPQEGLYNELQKDKMAEAYSEIGMKGERRRGKGHDGLYQGLSTATKDTYDALHMQALPPR

SEQ ID NO: 11 - protein, 483 aa, synthetic construct
  REGION 1..483: note = CAR-C11
EVQFVESGGGLVQPGGSLKLSCAASGVTFSEAWMDWVRQASGKGLEWVAEIRDKPNSYVTYYAESVKGRFTISRDDSKSTAYLQMNSLKTEDTAIYYCTGAMDYWGQGTLVTVSSGGGGSGGGGSGGGGSDIVMTQTPLSLSVTIGQPASISCKSSQSLLYSNGKTYLNWLLQKPGQSPKRLIYQVSKLDPGIPDRFSGSGSETDFTLKISRVEAEDVGIYYCMQGSSLPWTFGGGTKVEIKASSHFVPVFLPAKPTTTPAPRPPTPAPTIASQPLSLRPEACRPAAGGAVHTRGLDFACDFWVLVVVGGVLACYSLLVTVAFIIFWVKRGRKKLLYIFKQPFMRPVQTTQEEDGCSCRFPEEEEGGCELRVKFSRSADAPAYQQGQNQLYNELNLGRREEYDVLDKRRGRDPEMGGKPQRRKNPQEGLYNELQKDKMAEAYSEIGMKGERRRGKGHDGLYQGLSTATKDTYDALHMQALPPR

SEQ ID NO: 12 - protein, 486 aa, synthetic construct
  REGION 1..486: note = CAR-C12
EVKFEESGGGLVQPGGSIKLSCAASGVTFSEAWMDWVRQSPEKGLEWVAEIRDKPNSYVTYYAESVKGRFTISRDDSKSRVYLQMNNLRTEDTGIYYCTGAMDYWGQGTSVTVSSGSTGGGGSGGGGSGGGGSDIVMTQTPLSLSVTIGQPASISCKSSQSLLYSNGKTYLNWLQQRPGQSPKRLIYQVSKLDPGIPDRFSGSGSETDFTLKISRVEAEDLGIYYCMQGSSLPWTFGGGTKLEIKASSHFVPVFLPAKPTTTPAPRPPTPAPTIASQPLSLRPEACRPAAGGAVHTRGLDFACDFWVLVVVGGVLACYSLLVTVAFIIFWVKRGRKKLLYIFKQPFMRPVQTTQEEDGCSCRFPEEEEGGCELRVKFSRSADAPAYQQGQNQLYNELNLGRREEYDVLDKRRGRDPEMGGKPQRRKNPQEGLYNELQKDKMAEAYSEIGMKGERRRGKGHDGLYQGLSTATKDTYDALHMQALPPR

SEQ ID NO: 13 - protein, 468 aa, synthetic construct
  REGION 1..468: note = CAR-C13
EVQFVESGGGLVQPGGSLKLSCAASGVTFSEAWMDWVRQASGKGLEWVAEIRDKPNSYVTYYAESVKGRFTISRDDSKSTAYLQMNSLKTEDTAIYYCTGAMDYWGQGTLVTVSSGGGGSGGGGSGGGGSDIVMTQTPLSLSVTIGQPASISCKSSQSLLYSNGKTYLNWLLQKPGQSPKRLIYQVSKLDPGIPDRFSGSGSETDFTLKISRVEAEDVGIYYCMQGSSLPWTFGGGTKVEIKRSVTVSSAAAIEVMYPPPYLDNEKSNGTIIHVKGKHLCPSPLFPGPSKPFWVLVVVGGVLACYSLLVTVAFIIFWVRRDQRLPPDAHKPPGGGSFRTPIQEEQADAHSTLAKIRVKFSRSADAPAYQQGQNQLYNELNLGRREEYDVLDKRRGRDPEMGGKPQRRKNPQEGLYNELQKDKMAEAYSEIGMKGERRRGKGHDGLYQGLSTATKDTYDALHMQALPPR

SEQ ID NO: 14 - protein, 471 aa, synthetic construct
  REGION 1..471: note = CAR-C14
EVKFEESGGGLVQPGGSIKLSCAASGVTFSEAWMDWVRQSPEKGLEWVAEIRDKPNSYVTYYAESVKGRFTISRDDSKSRVYLQMNNLRTEDTGIYYCTGAMDYWGQGTSVTVSSGSTGGGGSGGGGSGGGGSDIVMTQTPLSLSVTIGQPASISCKSSQSLLYSNGKTYLNWLQQRPGQSPKRLIYQVSKLDPGIPDRFSGSGSETDFTLKISRVEAEDLGIYYCMQGSSLPWTFGGGTKLEIKRSVTVSSAAAIEVMYPPPYLDNEKSNGTIIHVKGKHLCPSPLFPGPSKPFWVLVVVGGVLACYSLLVTVAFIIFWVRRDQRLPPDAHKPPGGGSFRTPIQEEQADAHSTLAKIRVKFSRSADAPAYQQGQNQLYNELNLGRREEYDVLDKRRGRDPEMGGKPQRRKNPQEGLYNELQKDKMAEAYSEIGMKGERRRGKGHDGLYQGLSTATKDTYDALHMQALPPR

SEQ ID NO: 15 - protein, 478 aa, synthetic construct
  REGION 1..478: note = CAR-C15
EVQFVESGGGLVQPGGSLKLSCAASGVTFSEAWMDWVRQASGKGLEWVAEIRDKPNSYVTYYAESVKGRFTISRDDSKSTAYLQMNSLKTEDTAIYYCTGAMDYWGQGTLVTVSSGGGGSGGGGSGGGGSDIVMTQTPLSLSVTIGQPASISCKSSQSLLYSNGKTYLNWLLQKPGQSPKRLIYQVSKLDPGIPDRFSGSGSETDFTLKISRVEAEDVGIYYCMQGSSLPWTFGGGTKVEIKASSHFVPVFLPAKPTTTPAPRPPTPAPTIASQPLSLRPEACRPAAGGAVHTRGLDFACDFWVLVVVGGVLACYSLLVTVAFIIFWVRRDQRLPPDAHKPPGGGSFRTPIQEEQADAHSTLAKIRVKFSRSADAPAYQQGQNQLYNELNLGRREEYDVLDKRRGRDPEMGGKPQRRKNPQEGLYNELQKDKMAEAYSEIGMKGERRRGKGHDGLYQGLSTATKDTYDALHMQALPPR

SEQ ID NO: 16 - protein, 481 aa, synthetic construct
  REGION 1..481: note = CAR-C16
EVKFEESGGGLVQPGGSIKLSCAASGVTFSEAWMDWVRQSPEKGLEWVAEIRDKPNSYVTYYAESVKGRFTISRDDSKSRVYLQMNNLRTEDTGIYYCTGAMDYWGQGTSVTVSSGSTGGGGSGGGGSGGGGSDIVMTQTPLSLSVTIGQPASISCKSSQSLLYSNGKTYLNWLQQRPGQSPKRLIYQVSKLDPGIPDRFSGSGSETDFTLKISRVEAEDLGIYYCMQGSSLPWTFGGGTKLEIKASSHFVPVFLPAKPTTTPAPRPPTPAPTIASQPLSLRPEACRPAAGGAVHTRGLDFACDFWVLVVVGGVLACYSLLVTVAFIIFWVRRDQRLPPDAHKPPGGGSFRTPIQEEQADAHSTLAKIRVKFSRSADAPAYQQGQNQLYNELNLGRREEYDVLDKRRGRDPEMGGKPQRRKNPQEGLYNELQKDKMAEAYSEIGMKGERRRGKGHDGLYQGLSTATKDTYDALHMQALPPR

SEQ ID NO: 17 - protein, 479 aa, synthetic construct
  REGION 1..479: note = CAR-C23
EVQFVESGGGLVQPGGSLKLSCAASGVTFSEAWMDWVRQASGKGLEWVAEIRDKPNSYVTYYAESVKGRFTISRDDSKSTAYLQMNSLKTEDTAIYYCTGAMDYWGQGTLVTVSSGGGGSGGGGSGGGGSDIVMTQTPLSLSVTIGQPASISCKSSQSLLYSNGKTYLNWLLQKPGQSPKRLIYQVSKLDPGIPDRFSGSGSETDFTLKISRVEAEDVGIYYCMQGSSLPWTFGGGTKVEIKASSHFVPVFLPAKPTTTPAPRPPTPAPTIASQPLSLRPEACRPAAGGAVHTRGLDFACDIYIWAPLAGTCGVLLLSLVITLYCRSKRSRLLHSDYMNMTPRRPGPTRKHYQPYAPPRDFAAYRSRVKFSRSADAPAYQQGQNQLYNELNLGRREEYDVLDKRRGRDPEMGGKPQRRKNPQEGLYNELQKDKMAEAYSEIGMKGERRRGKGHDGLYQGLSTATKDTYDALHMQALPPR

SEQ ID NO: 18 - protein, 462 aa, synthetic construct
  REGION 1..462: note = CAR-C27
EVKFEESGGGLVQPGGSIKLSCAASGVTFSEAWMDWVRQSPEKGLEWVAEIRDKPNSYVTYYAESVKGRFTISRDDSKSRVYLQMNNLRTEDTGIYYCTGAMDYWGQGTSVTVSSGGGGSDIVMTQTPLSLSVTIGQPASISCKSSQSLLYSNGKTYLNWLQQRPGQSPKRLIYQVSKLDPGIPDRFSGSGSETDFTLKISRVEAEDLGIYYCMQGSSLPWTFGGGTKLEIKRSVTVSSAAAIEVMYPPPYLDNEKSNGTIIHVKGKHLCPSPLFPGPSKPFWVLVVVGGVLACYSLLVTVAFIIFWVRSKRSRLLHSDYMNMTPRRPGPTRKHYQPYAPPRDFAAYRSRVKFSRSADAPAYQQGQNQLYNELNLGRREEYDVLDKRRGRDPEMGGKPQRRKNPQEGLYNELQKDKMAEAYSEIGMKGERRRGKGHDGLYQGLSTATKDTYDALHMQALPPR

SEQ ID NO: 19 - protein, 472 aa, synthetic construct
  REGION 1..472: note = CAR-C28
EVKFEESGGGLVQPGGSIKLSCAASGVTFSEAWMDWVRQSPEKGLEWVAEIRDKPNSYVTYYAESVKGRFTISRDDSKSRVYLQMNNLRTEDTGIYYCTGAMDYWGQGTSVTVSSGGGGSDIVMTQTPLSLSVTIGQPASISCKSSQSLLYSNGKTYLNWLQQRPGQSPKRLIYQVSKLDPGIPDRFSGSGSETDFTLKISRVEAEDLGIYYCMQGSSLPWTFGGGTKLEIKASSHFVPVFLPAKPTTTPAPRPPTPAPTIASQPLSLRPEACRPAAGGAVHTRGLDFACDFWVLVVVGGVLACYSLLVTVAFIIFWVRSKRSRLLHSDYMNMTPRRPGPTRKHYQPYAPPRDFAAYRSRVKFSRSADAPAYQQGQNQLYNELNLGRREEYDVLDKRRGRDPEMGGKPQRRKNPQEGLYNELQKDKMAEAYSEIGMKGERRRGKGHDGLYQGLSTATKDTYDALHMQALPPR

SEQ ID NO: 20 - protein, 487 aa, synthetic construct
  REGION 1..487: note = CAR-C29
EVQFVESGGGLVQPGGSLKLSCAASGVTFSEAWMDWVRQASGKGLEWVAEIRDKPNSYVTYYAESVKGRFTISRDDSKSTAYLQMNSLKTEDTAIYYCTGAMDYWGQGTLVTVSSGGGGSGGGGSGGGGSGGGGSDIVMTQTPLSLSVTIGQPASISCKSSQSLLYSNGKTYLNWLLQKPGQSPKRLIYQVSKLDPGIPDRFSGSGSETDFTLKISRVEAEDVGIYYCMQGSSLPWTFGGGTKVEIKASSHFVPVFLPAKPTTTPAPRPPTPAPTIASQPLSLRPEACRPAAGGAVHTRGLDFACDFWVLVVVGGVLACYSLLVTVAFIIFWVRSKRSRLLHSDYMNMTPRRPGPTRKHYQPYAPPRDFAAYRSRVKFSRSADAPAYQQGQNQLYNELNLGRREEYDVLDKRRGRDPEMGGKPQRRKNPQEGLYNELQKDKMAEAYSEIGMKGERRRGKGHDGLYQGLSTATKDTYDALHMQALPPR

SEQ ID NO: 21 - protein, 477 aa, synthetic construct
  REGION 1..477: note = CAR-C30
EVKFEESGGGLVQPGGSIKLSCAASGVTFSEAWMDWVRQSPEKGLEWVAEIRDKPNSYVTYYAESVKGRFTISRDDSKSRVYLQMNNLRTEDTGIYYCTGAMDYWGQGTSVTVSSGGGGSGGGGSDIVMTQTPLSLSVTIGQPASISCKSSQSLLYSNGKTYLNWLQQRPGQSPKRLIYQVSKLDPGIPDRFSGSGSETDFTLKISRVEAEDLGIYYCMQGSSLPWTFGGGTKLEIKASSHFVPVFLPAKPTTTPAPRPPTPAPTIASQPLSLRPEACRPAAGGAVHTRGLDFACDFWVLVVVGGVLACYSLLVTVAFIIFWVRSKRSRLLHSDYMNMTPRRPGPTRKHYQPYAPPRDFAAYRSRVKFSRSADAPAYQQGQNQLYNELNLGRREEYDVLDKRRGRDPEMGGKPQRRKNPQEGLYNELQKDKMAEAYSEIGMKGERRRGKGHDGLYQGLSTATKDTYDALHMQALPPR

SEQ ID NO: 22 - protein, 21 aa, synthetic construct
  REGION 1..21: note = CD8ss
MALPVTALLLPLALLLHAARP

SEQ ID NO: 23 - protein, 115 aa, synthetic construct
  REGION 1..115: note = H3L3
EVQFVESGGGLVQPGGSLKLSCAASGVTFSEAWMDWVRQASGKGLEWVAEIRDKPNSYVTYYAESVKGRFTISRDDSKSTAYLQMNSLKTEDTAIYYCTGAMDYWGQGTLVTVSS

SEQ ID NO: 24 - protein, 115 aa, synthetic construct
  REGION 1..115: note = PP6373
EVKFEESGGGLVQPGGSIKLSCAASGVTFSEAWMDWVRQSPEKGLEWVAEIRDKPNSYVTYYAESVKGRFTISRDDSKSRVYLQMNNLRTEDTGIYYCTGAMDYWGQGTSVTVSS

SEQ ID NO: 25 - protein, 112 aa, synthetic construct
  REGION 1..112: note = H3L3
DIVMTQTPLSLSVTIGQPASISCKSSQSLLYSNGKTYLNWLLQKPGQSPKRLIYQVSKLDPGIPDRFSGSGSETDFTLKISRVEAEDVGIYYCMQGSSLPWTFGGGTKVEIK

SEQ ID NO: 26 - protein, 112 aa, synthetic construct
  REGION 1..112: note = PP6373
DIVMTQTPLSLSVTIGQPASISCKSSQSLLYSNGKTYLNWLQQRPGQSPKRLIYQVSKLDPGIPDRFSGSGSETDFTLKISRVEAEDLGIYYCMQGSSLPWTFGGGTKLEIK

SEQ ID NO: 27 - protein, 5 aa, synthetic construct
  REGION 1..5: note = GGGGS
GGGGS

SEQ ID NO: 28-29 - skipped (2 entries)

SEQ ID NO: 30 - protein, 4 aa, synthetic construct
  REGION 1..4: note = GGGS
GGGS

SEQ ID NO: 31 - protein, 5 aa, synthetic construct
  REGION 1..5: note = GSGGS
GSGGS

SEQ ID NO: 32 - protein, 39 aa, synthetic construct
  REGION 1..39: note = CD28
IEVMYPPPYLDNEKSNGTIIHVKGKHLCPSPLFPGPSKP

SEQ ID NO: 33 - protein, 57 aa, synthetic construct
  REGION 1..57: note = CD8
SHFVPVFLPAKPTTTPAPRPPTPAPTIASQPLSLRPEACRPAAGGAVHTRGLDFACD

SEQ ID NO: 34 - protein, 27 aa, synthetic construct
  REGION 1..27: note = CD28
FWVLVVVGGVLACYSLLVTVAFIIFWV

SEQ ID NO: 35 - protein, 24 aa, synthetic construct
  REGION 1..24: note = CD8
IYIWAPLAGTCGVLLLSLVITLYC

SEQ ID NO: 36 - protein, 42 aa, synthetic construct
  REGION 1..42: note = 41BB
KRGRKKLLYIFKQPFMRPVQTTQEEDGCSCRFPEEEEGGCEL

SEQ ID NO: 37 - protein, 41 aa, synthetic construct
  REGION 1..41: note = CD28
RSKRSRLLHSDYMNMTPRRPGPTRKHYQPYAPPRDFAAYRS

SEQ ID NO: 38 - protein, 37 aa, synthetic construct
  REGION 1..37: note = OX40
RRDQRLPPDAHKPPGGGSFRTPIQEEQADAHSTLAKI

SEQ ID NO: 39 - protein, 113 aa, synthetic construct
  REGION 1..113: note = CD3
RVKFSRSADAPAYQQGQNQLYNELNLGRREEYDVLDKRRGRDPEMGGKPQRRKNPQEGLYNELQKDKMAEAYSEIGMKGERRRGKGHDGLYQGLSTATKDTYDALHMQALPPR

SEQ ID NO: 40 - protein, 225 aa, synthetic construct
  REGION 1..225: note = RFP
MASSEDVIKEFMRFKVRMEGSVNGHEFEIEGEGEGRPYEGTQTAKLKVTKGGPLPFAWDILSPQFQYGSKAYVKHPADIPDYLKLSFPEGFKWERVMNFEDGGVVTVTQDSSLQDGEFIYKVKLRGTNFPSDGPVMQKKTMGWEASTERMYPEDGALKGEIKMRLKLKDGGHYDAEVKTTYMAKKPVQLPGAYKTDIKLDITSHNEDYTIVEQYERAEGRHSTGA

SEQ ID NO: 41 - DNA, 590 bp, synthetic construct
  misc_feature 1..590: note = IRES
  source 1..590: mol_type = other DNA
ccacctacatggggatccctcccccccccctaacgttactggccgaagccgcttggaataaggccggtgtgcgtttgtctatatgttattttccaccatattgccgtcttttggcaatgtgagggcccggaaacctggccctgtcttcttgacgagcattcctaggggtctttcccctctcgccaaaggaatgcaaggtctgttgaatgtcgtgaaggaagcagttcctctggaagcttcttgaagacaaacaacgtctgtagcgaccctttgcaggcagcggaaccccccacctggcgacaggtgcctctgcggccaaaagccacgtgtataagatacacctgcaaaggcggcacaaccccagtgccacgttgtgagttggatagttgtggaaagagtcaaatggctctcctcaagcgtattcaacaaggggctgaaggatgcccagaaggtaccccattgtatgggatctgatctggggcctcggtgcacatgctttacatgtgtttagtcgaggttaaaaaaacgtctaggccccccgaaccacggggacgtggttttcctttgaaaaacacgataataccatgacc

SEQ ID NO: 42 - protein, 10 aa, synthetic construct
  REGION 1..10: note = VH CDR1
GVTFSEAWMD

SEQ ID NO: 43 - protein, 19 aa, synthetic construct
  REGION 1..19: note = VH CDR2
EIRDKPNSYVTYYAESVKG

SEQ ID NO: 44 - protein, 4 aa, synthetic construct
  REGION 1..4: note = VH CDR3
AMDY

SEQ ID NO: 45 - protein, 16 aa, synthetic construct
  REGION 1..16: note = VL CDR1
KSSQSLLYSNGKTYLN

SEQ ID NO: 46 - protein, 7 aa, synthetic construct
  REGION 1..7: note = VL CDR2
QVSKLDP

SEQ ID NO: 47 - protein, 9 aa, synthetic construct
  REGION 1..9: note = VL CDR3
MQGSSLPWT

SEQ ID NO: 48 - protein, 854 aa, synthetic construct
  REGION 1..854: note = C31
EVKFEESGGGLVQPGGSIKLSCAASGVTFSEAWMDWVRQSPEKGLEWVAEIRDKPNSYVTYYAESVKGRFTISRDDSKSRVYLQMNNLRTEDTGIYYCTGAMDYWGQGTSVTVSSGGGGSDIVMTQTPLSLSVTIGQPASISCKSSQSLLYSNGKTYLNWLQQRPGQSPKRLIYQVSKLDPGIPDRFSGSGSETDFTLKISRVEAEDLGIYYCMQGSSLPWTFGGGTKLEIKASSHFVPVFLPAKPTTTPAPRPPTPAPTIASQPLSLRPEACRPAAGGAVHTRGLDFACDFWVLVVVGGVLACYSLLVTVAFIIFWVRSKRSRLLHSDYMNMTPRRPGPTRKHYQPYAPPRDFAAYRSRVKFSRSADAPAYQQGQNQLYNELNLGRREEYDVLDKRRGRDPEMGGKPQRRKNPQEGLYNELQKDKMAEAYSEIGMKGERRRGKGHDGLYQGLSTATKDTYDALHMQALPPRGSGATNFSLLKQAGDVEENPGPMEDFNMESDSFEDFWKGEDLSNYSYSSTLPPFLLDAAPCEPESLEINKYFVVIIYALVFLLSLLGNSLVMLVILYSRVGRSVTDVYLLNLALADLLFALTLPIWAASKVNGWIFGTFLCKVVSLLKEVNFYSGILLLACISVDRYLAIVHATRTLTQKRYLVKFICLSIWGLSLLLALPVLLFRRTVYSSNVSPACYEDMGNNTANWRMLLRILPQSFGFIVPLLIMLFCYGFTLRTLFKAHMGQKHRAMRVIFAVVLIFLLCWLPYNLVLLADTLMRTQVIQETCERRNHIDRALDATEILGILHSCLNPLIYAFIGQKFRHGLLKILAIHGLISKDSLPKDSRPSFVGSSSGHTSTTL

SEQ ID NO: 49 - protein, 822 aa, synthetic construct
  REGION 1..822: note = C32
EVKFEESGGGLVQPGGSIKLSCAASGVTFSEAWMDWVRQSPEKGLEWVAEIRDKPNSYVTYYAESVKGRFTISRDDSKSRVYLQMNNLRTEDTGIYYCTGAMDYWGQGTSVTVSSGGGGSDIVMTQTPLSLSVTIGQPASISCKSSQSLLYSNGKTYLNWLQQRPGQSPKRLIYQVSKLDPGIPDRFSGSGSETDFTLKISRVEAEDLGIYYCMQGSSLPWTFGGGTKLEIKASSHFVPVFLPAKPTTTPAPRPPTPAPTIASQPLSLRPEACRPAAGGAVHTRGLDFACDFWVLVVVGGVLACYSLLVTVAFIIFWVRSKRSRLLHSDYMNMTPRRPGPTRKHYQPYAPPRDFAAYRSRVKFSRSADAPAYQQGQNQLYNELNLGRREEYDVLDKRRGRDPEMGGKPQRRKNPQEGLYNELQKDKMAEAYSEIGMKGERRRGKGHDGLYQGLSTATKDTYDALHMQALPPRGSGATNFSLLKQAGDVEENPGPMCHQQLVISWFSLVFLASPLVAIWELKKDVYVVELDWYPDAPGEMVVLTCDTPEEDGITWTLDQSSEVLGSGKTLTIQVKEFGDAGQYTCHKGGEVLSHSLLLLHKKEDGIWSTDILKDQKEPKNKTFLRCEAKNYSGRFTCWWLTTISTDLTFSVKSSRGSSDPQGVTCGAATLSAERVRGDNKEYEYSVECQEDSACPAAEESLPIEVMVDAVHKLKYENYTSSFFIRDIIKPDPPKNLQLKPLKNSRQVEVSWEYPDTWSTPHSYFSLTFCVQVQGKSKREKKDRVFTDKTSATVICRKNASISVRAQDRYYSSSWSEWASVPCS

SEQ ID NO: 50 - protein, 328 aa, synthetic construct
  REGION 1..328: note = p40
MCHQQLVISWFSLVFLASPLVAIWELKKDVYVVELDWYPDAPGEMVVLTCDTPEEDGITWTLDQSSEVLGSGKTLTIQVKEFGDAGQYTCHKGGEVLSHSLLLLHKKEDGIWSTDILKDQKEPKNKTFLRCEAKNYSGRFTCWWLTTISTDLTFSVKSSRGSSDPQGVTCGAATLSAERVRGDNKEYEYSVECQEDSACPAAEESLPIEVMVDAVHKLKYENYTSSFFIRDIIKPDPPKNLQLKPLKNSRQVEVSWEYPDTWSTPHSYFSLTFCVQVQGKSKREKKDRVFTDKTSATVICRKNASISVRAQDRYYSSSWSEWASVPCS

SEQ ID NO: 51 - protein, 22 aa, synthetic construct
  REGION 1..22: note = P2A
GSGATNFSLLKQAGDVEENPGP

SEQ ID NO: 52 - protein, 21 aa, synthetic construct
  REGION 1..21: note = T2A
GSGEGRGSLLTCGDVEENPGP

SEQ ID NO: 53 - protein, 360 aa, synthetic construct
  REGION 1..360: note = CXCR2
MEDFNMESDSFEDFWKGEDLSNYSYSSTLPPFLLDAAPCEPESLEINKYFVVIIYALVFLLSLLGNSLVMLVILYSRVGRSVTDVYLLNLALADLLFALTLPIWAASKVNGWIFGTFLCKVVSLLKEVNFYSGILLLACISVDRYLAIVHATRTLTQKRYLVKFICLSIWGLSLLLALPVLLFRRTVYSSNVSPACYEDMGNNTANWRMLLRILPQSFGFIVPLLIMLFCYGFTLRTLFKAHMGQKHRAMRVIFAVVLIFLLCWLPYNLVLLADTLMRTQVIQETCERRNHIDRALDATEILGILHSCLNPLIYAFIGQKFRHGLLKILAIHGLISKDSLPKDSRPSFVGSSSGHTSTTL